European Patent Application EP 4 768 604 A1, published July 1, 2026. Title: METHOD OF DETECTING THE PRESENCE OF EXONS 5 AND 6 OF ANRIL IN A SUBJECT, KIT, SETS OF OLIGONUCLEOTIDES AND THEIR USES. Applicant: CNRS. The sequence listing filed with the application follows.

SEQUENCE LISTING (7 sequences)

SEQ ID NO: 1 - DNA, 20 bp, synthetic construct
  source 1..20: mol_type = other DNA
tgtcccttttgatgagaaga

SEQ ID NO: 2 - DNA, 18 bp, synthetic construct
  source 1..18: mol_type = other DNA
ccaaatagatctccccgg

SEQ ID NO: 3 - DNA, 45 bp, synthetic construct
  source 1..45: mol_type = other DNA
acatatatctggtggccagaaaacacctcattctgattcaacagc

SEQ ID NO: 4 - DNA, 43 bp, synthetic construct
  source 1..43: mol_type = other DNA
aggagaattttcttggaaagagaggaaagcagtactgactcgg

SEQ ID NO: 5 - DNA, 24 bp, synthetic construct
  source 1..24: mol_type = other DNA
catcactgttaggtgtgctggaat

SEQ ID NO: 6 - RNA, 42 nt, synthetic construct
  source 1..42: mol_type = other RNA
taatttctactaagtgtagatttggaaagagagggttcaagc

SEQ ID NO: 7 - DNA, 11 bp, synthetic construct
  source 1..11: mol_type = other DNA
ttattattatt